European Patent Application EP 4 166 647 A1, published April 19, 2023. Title: METHOD FOR PRODUCING PROTEIN. Applicant: Ajinomoto Co., Inc. The sequence listing filed with the application follows.

SEQUENCE LISTING (74 sequences)

SEQ ID NO: 1 - DNA, 40 bp, Artificial Sequence
  primer
cggtacccggggatccccttcttgccagcacactgctccg

SEQ ID NO: 2 - DNA, 40 bp, Artificial Sequence
  primer
agctgcgaggtcaacggctaagcgccagtttggtgaatcc

SEQ ID NO: 3 - DNA, 40 bp, Artificial Sequence
  primer
aactggcgcttagccgttgacctcgcagctggcacgggat

SEQ ID NO: 4 - DNA, 40 bp, Artificial Sequence
  primer
cgactctagaggatccgccaagggatccgtgagatcgcat

SEQ ID NO: 5 - DNA, 40 bp, Artificial Sequence
  primer
cggtacccggggatcttggggcacagagacaacagggtca

SEQ ID NO: 6 - DNA, 40 bp, Artificial Sequence
  primer
acctgactcgaccggagatagcgtgagcacactgagcagg

SEQ ID NO: 7 - DNA, 40 bp, Artificial Sequence
  primer
gcttgttgacctcgccaacacgctacctcttccacagtag

SEQ ID NO: 8 - DNA, 40 bp, Artificial Sequence
  primer
cgactctagaggatcgagctgattgagcatgctaacgcag

SEQ ID NO: 9 - DNA, 25 bp, Artificial Sequence
  primer
ccggtcgagtcaggtattcatatca

SEQ ID NO: 10 - DNA, 25 bp, Artificial Sequence
  primer
gcgaggtcaacaagcctcaaaccct

SEQ ID NO: 11 - DNA, 40 bp, Artificial Sequence
  primer
cggtacccggggatcagcaaccccaccgtaatctcaaggt

SEQ ID NO: 12 - DNA, 40 bp, Artificial Sequence
  primer
ccgatctgaattgacattcggatggactttttgaaggcca

SEQ ID NO: 13 - DNA, 40 bp, Artificial Sequence
  primer
tcggcgttcacttatgaggttgacttgatagtcgatcgct

SEQ ID NO: 14 - DNA, 40 bp, Artificial Sequence
  primer
cgactctagaggatcgttattgctgttgctgttgtggttg

SEQ ID NO: 15 - DNA, 40 bp, Artificial Sequence
  primer
cggtacccggggatccatagcctcatgaccaatgaccggt

SEQ ID NO: 16 - DNA, 40 bp, Artificial Sequence
  primer
ccgatctgaattgacgtcgatgaagtcgtcgggggtatgt

SEQ ID NO: 17 - DNA, 40 bp, Artificial Sequence
  primer
tcggcgttcacttatcggctcaatatgcaataggtgttcc

SEQ ID NO: 18 - DNA, 40 bp, Artificial Sequence
  primer
cgactctagaggatctagggctaaccagcagggtaccgcc

SEQ ID NO: 19 - DNA, 40 bp, Artificial Sequence
  primer
cggtacccggggatctagacgttagaactctccccactgt

SEQ ID NO: 20 - DNA, 40 bp, Artificial Sequence
  primer
ccgatctgaattgaccttgccgcttgaagttgtatgaaat

SEQ ID NO: 21 - DNA, 40 bp, Artificial Sequence
  primer
tcggcgttcacttatgtgttgcattcaaagatggctgcct

SEQ ID NO: 22 - DNA, 40 bp, Artificial Sequence
  primer
cgactctagaggatccggcgtttgagctcctggagtaaga

SEQ ID NO: 23 - DNA, 40 bp, Artificial Sequence
  primer
cggtacccggggatcaattccgacagtgtcgtgctccagc

SEQ ID NO: 24 - DNA, 40 bp, Artificial Sequence
  primer
ccgatctgaattgacggcgggcgattgataatgatgttgt

SEQ ID NO: 25 - DNA, 40 bp, Artificial Sequence
  primer
tcggcgttcacttatctagcgacgaggtcacgattatgag

SEQ ID NO: 26 - DNA, 40 bp, Artificial Sequence
  primer
cgactctagaggatcacaagaccttcaatctctccaggag

SEQ ID NO: 27 - DNA, 40 bp, Artificial Sequence
  primer
cggtacccggggatctacacgcaagggaagaagtaagagc

SEQ ID NO: 28 - DNA, 40 bp, Artificial Sequence
  primer
ccgatctgaattgacgatggccaaccaacgctaatgtatc

SEQ ID NO: 29 - DNA, 40 bp, Artificial Sequence
  primer
tcggcgttcacttatatcggttgacgggttgctgaaatgc

SEQ ID NO: 30 - DNA, 39 bp, Artificial Sequence
  primer
cgactctagaggatctagtcgcaggacggaatcgaacag

SEQ ID NO: 31 - DNA, 25 bp, Artificial Sequence
  primer
gtcaattcagatcggctgccgcctg

SEQ ID NO: 32 - DNA, 25 bp, Artificial Sequence
  primer
ataagtgaacgccgagtcagtacta

SEQ ID NO: 33 - DNA, 26 bp, Artificial Sequence
  primer
cccagtcacgacgttgtaaaacgacg

SEQ ID NO: 34 - DNA, 26 bp, Artificial Sequence
  primer
caggaaacagctatgaccatgattac

SEQ ID NO: 35 - DNA, 40 bp, Artificial Sequence
  primer
ccgatctgaattgacagatagcgtgagcacactgagcagg

SEQ ID NO: 36 - DNA, 40 bp, Artificial Sequence
  primer
tcggcgttcacttatcaacacgctacctcttccacagtag

SEQ ID NO: 37 - DNA, 40 bp, Artificial Sequence
  primer
cggtacccggggatcagcgcagaccaatgccagaggagaa

SEQ ID NO: 38 - DNA, 25 bp, Artificial Sequence
  primer
gcgcgagttgcgcgatgaaatttat

SEQ ID NO: 39 - DNA, 40 bp, Artificial Sequence
  primer
tcgcgcaactcgcgctgctatgcagttgatgctactgtgt

SEQ ID NO: 40 - DNA, 30 bp, Artificial Sequence
  primer
agttgctaaatgatcaagaagcttcacttt

SEQ ID NO: 41 - DNA, 40 bp, Artificial Sequence
  primer
gttgaagctcagcaaattggtacttataccgctgaaaccc

SEQ ID NO: 42 - DNA, 40 bp, Artificial Sequence
  primer
gacgagctggacttcctgagcaccagctgttgccagcaag

SEQ ID NO: 43 - DNA, 30 bp, Artificial Sequence
  primer
taaattttcacttctttcttcgcctattga

SEQ ID NO: 44 - DNA, 45 bp, Artificial Sequence
  primer
ccgatctgaattgacccgaaaacggtaaggcgtagttatagaaat

SEQ ID NO: 45 - DNA, 40 bp, Artificial Sequence
  primer
tcggcgttcacttattgctatgcagttgatgctactgtgt

SEQ ID NO: 46 - DNA, 40 bp, Artificial Sequence
  primer
tgtcatctggatgtcctgagcaccagctgttgccagcaag

SEQ ID NO: 47 - DNA, 25 bp, Artificial Sequence
  primer
tagatcagctttgagtgcagcaaaa

SEQ ID NO: 48 - DNA, 27 bp, Artificial Sequence
  primer
gcttgtttgagaatacatgaggttgcc

SEQ ID NO: 49 - DNA, 40 bp, Artificial Sequence
  primer
tattctcaaacaagccctctttctcgccctttcttctcaa

SEQ ID NO: 50 - DNA, 40 bp, Artificial Sequence
  primer
cgactctagaggatcaaccgtcgatcagaaggagcgcaat

SEQ ID NO: 51 - DNA, 25 bp, Artificial Sequence
  primer
gaagtccagctcgtcgagtctggtg

SEQ ID NO: 52 - DNA, 37 bp, Artificial Sequence
  primer
agaagtgaaaatttatttaccaggagacaaggacaga

SEQ ID NO: 53 - DNA, 25 bp, Artificial Sequence
  primer
gacatccagatgacacagtcccctt

SEQ ID NO: 54 - DNA, 40 bp, Artificial Sequence
  primer
ctcaaagctgatctaacactcaccacggttgaaggactta

SEQ ID NO: 55 - DNA, 40 bp, Artificial Sequence
  primer
agatagggttgagtggatggccaaccaacgctaatgtatc

SEQ ID NO: 56 - DNA, 40 bp, Artificial Sequence
  primer
tagctagagcttggcatcggttgacgggttgctgaaatgc

SEQ ID NO: 57 - DNA, 21 bp, Artificial Sequence
  primer
cactcaaccctatctcggtct

SEQ ID NO: 58 - DNA, 25 bp, Artificial Sequence
  primer
gccaagctctagctagaggtcgacg

SEQ ID NO: 59 - DNA, 1988 bp, Talaromyces cellulolyticus
atggcaaaccctcctcacggtggtatcctcaaggacttggtggcccgcgatgcccctcgtcatgccgagctcgaggctgaagctgccaccctacctgctattcttctcacagaacgccaattgtgtgatttggagttgattatgaatggtggtttcagtcctcttgaaggtaagtctttttgtcgcacgcgatcgagaagattattagctaacatttttcttctataggtttcatgaacgagaaagattacgatgggtatgcaacatatcttgcgcgcgcagtgaaaggaacaattttctgactgacttagtgttgtcgccgaatctcgcctcgccgatggcaaccttttctccatgcccattactctcgatgcctctggcgaaaccattaaagaccttggcttgaaggctggatctcgtgtcacattacgcgatttccgtgacgaccgcaaccttgctattttgaccattgatgatatctaccgccctgacaagtgagtcctgcaatcagcttgtgcgacgaaacatgctgaccccttttaccaggacgaaagaagcccagctcgtctttggaggtgacgaagagcaccccgctatcgtatatctcaataccaaggttcaggagttctacattggaggaaaggtcgaagctgttaacaaacttgcccactacgactatgtcgctctccgatgtgagttactattcaacagagacaatagtacatagactaaccatgtagacactcccgctgaattgcgcacacacttcgacaagctcggctggacccgagttgttgctttccagaccaggtatgctaaaagcagacgataggagttatttgaatgtcactgacactagtagaaaccccatgcatcgtgctcaccgtgaattgaccgtccgcgctgcccgtgctcgtcaagccaatgtgctcatccaccccgtcgtcggtctcaccaagcccggtgacattgaccacttcacccgtgtccgtgtctaccaagcccttcttcctcgttaccccaacggcatggctgtcctcggtcttttgcctcttgctatgcgtatgggtggtcctcgtgaggccatctggcacgccattatccgtaagaaccacggtgccacccacttcattgtcggacgtgaccacgccggtcccggaaagaactccaagggtgtcgaattttacggtccttacgatgctcagcatgctgttgagaagtacaggtctgagttgggtattgaggtggttgaattccagcaggttacctacctgcctgataccgacgagtacaagcctgttaatgaggtttctgccggtgtaaagactcttgatatctctggtactgagctcaggagacgtcttcgctcgggtgctcacatcccagagtggttctcttaccctgaggtcatcaaggttctccgcgagtccaacccccctcgcaatgctcaaggtttcaccgtcttcctcactggataccagaactctggcaaggacgccattgcccgcgctcttcaagtgactctcaaccagcaaggtggccggtccgtctcgctcttgttgggagagaccgtccgtcacgagctttcctcagagcttggtttcagccgcgaagaccgcgacaaaaacattcaacgtattgcctttgtcgctgccgagctcaccaaggccggtgctgccgttatcgctgcacccatcgctccttacgaatcatcccgaaaggctgccaaagacaccatctccgcagtcggcacattcattctcgtccacgtcgccacccctcttgagtactgcgagaagaccgacaagcgcggaatctacgcgaaggcccgccgcggcgagatcaagggcttcactggtgtcgatgacccatacgaggctcccgccaaggccgacctcgtggtcgacgttgagaagcagagtgtccgcagtatcgtgcacgagattgtcttgattctcgagagccagggattcctcgatcggtcttag

SEQ ID NO: 60 - DNA, 1589 bp, Talaromyces cellulolyticus
atgaagggcgtcctcagcctttcgctgctgccgttgttgacggttgcgtcaccggtgatgccgcgcaccatccacaacgacgctgctcccattctctcttcgtccaacgccgttgaggtcccagattcatatatcattgtctttaaagaccatgtagattctgcttctgccgcagcccatcataactgggtgcaagacattcacagccaacacaccgagctccgaaagcggtctcaattcccattcgctgacaatgcctttgccggtctcaaacacacttttgacattgccggcagcttccttggttactcaggacacttcgaagagaatgtcattgaggccattcgccgacaccccgatgtgagttatccgcacgtgccctactcctaaggcaatgactaatacgcatctccacctataggttgattacatcgagaaggattctcttgtccacaccatggaagatcccgcccttgagaagaacgccccatggggtttggctcgtatttcgcaccgtgagagcttgagcttcggaagcttcaacaagtacttgtacgctgccgacggcggtgaaggtgttgacgtttatgtcattgacactggtaccaacatcgaccacgtcgacttcgagggtcgtgcttcctggggcaagaccatccccactgacgatgaggatgttgatggcaatggtcacggtactcactgctccggaactattgcgggcaagaagtacggtgttgccaagaaggccaatgtctacgctgtcaaggtcttgaagtctaacggttctggaaccatgtccgatgtcgttcagggtgtcgaatgggctgctactcagcacatcaagaaggtcaaggacgccaaggccggaaaagccaagggcttcaagggtagcgctgcgaacatgagtctcggtggtggcaagtccgtcactcttgacaaggctgtcaatgctgctgttgatgctggtatccacttcgctgtcgctgctggcaacgacaacgccgactcctgcaactactcccctgccgccgctgagaaggccgtcaccgtcggagcctcgaccttggccgatgagcgtgcttacttctccaactacggcaagtgcaacgacatctttgctcctggtctgaacattctctctacctggatcggcagcaagtacgccgtcaacaccatctccggtacctccatggcttctcctcacattgctggtcttttggcctacttcctctctctccagcctgccagtgactccgccttcgctgttgccgagattactcccaagaagttgaaggagaacctcattgctattggtacccagggcgctcttactgatgttccctctgacaccactaacgtaagttgactctgttagtctttcaatgcattatcaactaacaactgtgtcatagattctcgcctggaacggtggtggctcagccaactacaccgacatcattgcccaaggtggttacaagaccaagacactcagcaacgaagttgacgaattgatcaacaagttggaggtcgtgaacgaggaactcggtgccatctacagccacatcaaggatgccattgccgcataa

SEQ ID NO: 61 - DNA, 3534 bp, Talaromyces cellulolyticus
ccggtcgagtcaggtattcatatcatccattcatggattgttatctgtgaacacaacgccaacgttgcaaaatccggccatttgatggcacggtttaaatgtcccttgctcattggggatgaaaatattcaacgtaagttctacatccttggctatcaatgtcgcttgccgggtcaaatcattcaatactgtcctggacagtcctctttccaaccggtggagtaatctaggcaaggttcattcggcaagtttcctaggcatcatggttccaaaaagtgaaaaaagagactgggagaatcatatatccatctcagcctatatggctacgtcttgaacagtgaccttgccataaatggcgacatgaagtagggttagggctagggcttttctcaggttatggcatcataagtcttggcagggacgttaatgttagcatgcaatcacgcaagccgccaagccgatgtcgtgattgcttttctgtctggaactggcagccgctaaactgtaatgggattcaccaaactggcgcttagccagatatagtctagtgtctgatctcttgtttaaaaatttcgcaatgtattgattgtattcaaatgtagtaagtgtattgcgattgtatacagattcgaagtaataaattgcgccagtcgactgaattgttacacattttcttaaaggcacaaatagttgaattggcattacttggcgagattgaaagagacgtttgagctgatgtggcagtcgtcatggtgtaattttgggcgtattccacgtaatcaattcccttggtcaatgcatatctggccaataaaattaacgcgtccaccacggatagttgattaccttatcgataaaagtgggatgtaagtaatttaaggaaccgtaccacagtgatacatacagcaaccaccatctcttccgacatcagctccgattatttcttcttcattccttttattttgaactcattctttttctctttcttcttccttgatatatttgtttgttaattctctcttcatatcaataaaaatggcaaaccctcctcacggtggtatcctcaaggacttggtggcccgcgatgcccctcgtcatgccgagctcgaggctgaagctgccaccctacctgctattcttctcacagaacgccaattgtgtgatttggagttgattatgaatggtggtttcagtcctcttgaaggtaagtctttttgtcgcacgcgatcgagaagattattagctaacatttttcttctataggtttcatgaacgagaaagattacgatgggtatgcaacatatcttgcgcgcgcagtgaaaggaacaattttctgactgacttagtgttgtcgccgaatctcgcctcgccgatggcaaccttttctccatgcccattactctcgatgcctctggcgaaaccattaaagaccttggcttgaaggctggatctcgtgtcacattacgcgatttccgtgacgaccgcaaccttgctattttgaccattgatgatatctaccgccctgacaagtgagtcctgcaatcagcttgtgcgacgaaacatgctgaccccttttaccaggacgaaagaagcccagctcgtctttggaggtgacgaagagcaccccgctatcgtatatctcaataccaaggttcaggagttctacattggaggaaaggtcgaagctgttaacaaacttgcccactacgactatgtcgctctccgatgtgagttactattcaacagagacaatagtacatagactaaccatgtagacactcccgctgaattgcgcacacacttcgacaagctcggctggacccgagttgttgctttccagaccaggtatgctaaaagcagacgataggagttatttgaatgtcactgacactagtagaaaccccatgcatcgtgctcaccgtgaattgaccgtccgcgctgcccgtgctcgtcaagccaatgtgctcatccaccccgtcgtcggtctcaccaagcccggtgacattgaccacttcacccgtgtccgtgtctaccaagcccttcttcctcgttaccccaacggcatggctgtcctcggtcttttgcctcttgctatgcgtatgggtggtcctcgtgaggccatctggcacgccattatccgtaagaaccacggtgccacccacttcattgtcggacgtgaccacgccggtcccggaaagaactccaagggtgtcgaattttacggtccttacgatgctcagcatgctgttgagaagtacaggtctgagttgggtattgaggtggttgaattccagcaggttacctacctgcctgataccgacgagtacaagcctgttaatgaggtttctgccggtgtaaagactcttgatatctctggtactgagctcaggagacgtcttcgctcgggtgctcacatcccagagtggttctcttaccctgaggtcatcaaggttctccgcgagtccaacccccctcgcaatgctcaaggtttcaccgtcttcctcactggataccagaactctggcaaggacgccattgcccgcgctcttcaagtgactctcaaccagcaaggtggccggtccgtctcgctcttgttgggagagaccgtccgtcacgagctttcctcagagcttggtttcagccgcgaagaccgcgacaaaaacattcaacgtattgcctttgtcgctgccgagctcaccaaggccggtgctgccgttatcgctgcacccatcgctccttacgaatcatcccgaaaggctgccaaagacaccatctccgcagtcggcacattcattctcgtccacgtcgccacccctcttgagtactgcgagaagaccgacaagcgcggaatctacgcgaaggcccgccgcggcgagatcaagggcttcactggtgtcgatgacccatacgaggctcccgccaaggccgacctcgtggtcgacgttgagaagcagagtgtccgcagtatcgtgcacgagattgtcttgattctcgagagccagggattcctcgatcggtcttaggtttgcttgtgaacaaaaccaaaagaaatgagttatgcaattggtttagggtaatgaatgtgcttgatatggaagcaatgtgcatacagattaggagctacatagaggcgttaatctagttatttgcatcccttttcgccctgtagatatagtttgtggagtatgatcaacgtggggttgatctgataaagtcgtccatatcggagatttatccgatatccaatatccgattatcgcaattggccattgaactagagtattcgtcatctactgacgatttgtacatatgtacttagtttcaatcccccttcttcctccaatccatctggtgcaattatagatagagaggaaagaaaatgacccaatcaatccaccacatagcccaaaccggcttctcagacgcctcatcctacgacaaacacagaccaacctacaccgcgcacgaaacagatctgattctaaaccgcacgaatgtcgcgaaccgtaagggtttgaggcttgttgacctcgc

SEQ ID NO: 62 - DNA, 2858 bp, Talaromyces cellulolyticus
gtcaattcagatcggctgccgcctgcgccccaggtgacgtcgatgaaagctgggcctaggtcgtgcatgcggtccatacggtcgtataagttctggacaccttgggcggtctttggggggaagtattcgaaggaaattccaggtcggccggtggccgcctgttcttggagcttttgcccgacatgcatgttgataggtcggtcaattgtctgctttttcaatatcttctcggtatgatgtagcttgcagaacccaagttatgtagttcaattgcaaaatcaagtctgatcaagaccgaaactcaatcccggagcactgaggttcgcactaattgatcaagggtacaagaatgaggggcacaatgaaagcagtcttgaaaatgacaggcagagaaattgaaagaaaggagaagagaggacctccgggacaggagaaatgaaagcaacaaaaccccgaacaagctggagagaagttaaagggagcagcttggtcaccggcaatggatgctcatcataaaaaaggaccctaaacccgttatcggagtccggagaaatgacgctaattcggatttggaagtccccgccaatcgtgggaaattctcgaagcagacaatttgctcgtgacaatcagccagcaatgagagggagactgaaaaatatgtatttacactcaaagaatccgatactgctattaggatcagtgtttttcttataagcaaatgagcgttggacgtggaaaatgaggaatcctcagtccctatactcggtcagcgacggaggggtgcgtgatcggccaatcacagcctattattttatcaacatctgattggctacttccgataagagcgaaatatgcccctccttgcaatttttaccatcaacgctaacagcaacactcaacaaaccattcaatcttgatactcgctcccattagtcaccacgcaggacaacacaacacgacatcgcatctcagctttgaccattcccgccgcaagcgattcgctgtcacaaacgccagataccccaacatggctgcccctccctccgccgatcaggactacaagaccaatctgttgtctttgctgatagccaacgatgcgctcgcatttggcacgttcacattgaaatctggtcgccagtcgccgtattttttgacctcgagtcgtctttatactgcgcctctgctgcgccaggtgtcggccgcgttcgcgaataccatctcgtccccgccttttgtgaatatagctgcagatggcagcattaccccgaactttgacattgtttttgggtatgttaccctattattcgtgcgcctgatatgcgtgtactgatttacttcaaatagccccgcctacaaaggaatccccgaatgcgtcggtgttgtcaacgagctcgctacccgggatgcgctcgccggtaccaagacatgggacaacatcagctactccttcaaccgcaaagaagccaaagaccacggcgaagggggtaacatcgtcggtgcgcctctcaagggaaaacgtgttttgatcgttgacgacgtcatcaccgctggtaccgcgctgcgtgaagctgtcggcattattcaaaaggaaggcggaaccgttgccggtgttgtgttgctgttcgatcgtcaggaacgggtcagtgatacggagcagaagagtgccattggagccgcggagagggaccttggaggcgatattcctatccgtgcggtgttggtattccaggatttgattgataagcttggagataagattggtcaggaggaggtgcgcaggttggaagagtaccggaacacgtacaaggctcaataaatggctgctgtgggatgaaatgggtatattaacgatttatgctaaaaatggctgggtggaatactgcgaaataaatataaatcagcttgaaggatgtatttttagcgcaaagtgatagaattttctatgtaaatagtttgtacaataggattactactttatatgcgttatgcgtatacatttctaaagtgtaaccagtttagctgggagtacaattttaacactcttccatcaatcaggttccagatcagttttctatctacaatcatgactccccagtctctactcctttcaagaatgacgcgttatgttccaagctcccctggttgatggcggtaacccgatatattctagccaggtcaggtcctagtgtgaggactaacacaggcacgtccagtatcgtagcaaatagaatatcagcatatataagtcccctttcccggaccttgctcgagtcagtgactagcaggtacgtacgtacccatcagactatctactatctactatgtacggagtatatagtcggtacttgacgcaaggcgagtctgatagagggacaatatgcagttctgtagccaatcaatcgcggatggcagaccctcgatcgtcattgtggatctttagcttccttatgggcggggcggtggttatttcagagccatttagccaatcatacatcgtagtccgaaagtctaggattatataggctagaccaatctactgtcaaccggtaaagcgggtctctagtctttatcccgacctcctctctttctctttctccgattcgaatgtgacacatacatctgatcaattgataagaatacggattgccgtgtacgtgggctgacagagctgagataaaatatcctggatgtgatatgtggcgcatccagtaccgacactgtgacaggatccgtgtactacaattcattcatcgatcgttggctaggcaaaaagtaggcaaggtttgcagatcgatatcccggtacctggctaaaatcgagacccatctacatatagtactgactcggcgttcacttat

SEQ ID NO: 63 - DNA, 1100 bp, Talaromyces cellulolyticus
tgctatgcagttgatgctactgtgttctaaaataattgatagggttagggtcgggtataaggcgatgcaatgtatcaattatcacgagaaataatgcagaaaaacacaattccccgtatctgttgattcttaaacaatctgatcaccaatttgtagaaagaaacgattataaggtgccatggtaatgctggagtttacacaggatactacttgttctgttcattacaatgaaccgtaattgcattctgttttgaccactcaacaaatcctacacaaaagtaagtggacttcagtgctcgctctacgcaagtaaatacttggcatatatggcctcgtatattcttacaatgaggtaaattccgatagattactgcccaactagtcaatcttaaatccttaagagatacagggggaggcggaagtacctgaaaccacgtaataagacgttcagggtcatgtgaatgtatgtagtatccatgtccaatacaattgataatagtatccagtattatatctcattcaggtaagcgccacgcgattcttcagatctacttaactgccgactcgccaaacgaaacaacgtttattcgtgaccccagaaaatcaccgcggagttgcggaggaccagtttgtacaatgcaccgaaccaagcgttggtcatttttctggaaatgggccaaacgttagaagtgattggtcagagctacatctgaaggtgaagcaatttccggtatgcatacatgacagcaagcttacctaccaagaccaagttattccccagcatttgccccatacttggctttaatattgtgggatagcaaacaatatccacaacactgatgataactaaactacaaatctgacgttacttcagactactcacgtgtcaaaagcagttagcgaggatcaagtcttttagtctggtcattaacaaacgcaatttcgcaacccgataatccgcgatgataatatagcgactccaaggtcgtatttatattcaatcaattccccccaatttggaatggatttttggaatcatcgcatgccaggacaatcagtgaaacagtgacaaagtgaagcttcttgatcatttagcaact

SEQ ID NO: 64 - DNA, 78 bp, Talaromyces cellulolyticus
atgtctgccttgaactctttcaatatgtacaagagcgccctcatcttgggctccttgctggcaacagctggtgctcag

SEQ ID NO: 65 - DNA, 1356 bp, Homo sapiens
gaagtccagctcgtcgagtctggtggtggcttggtccaacccggtggatccttacgtctctcttgtgcagctagcggtttcaacatcaaggacacctacatccattgggttcgtcaagctcctggcaaaggtttggaatgggttgcgcgtatctaccctacgaacggttacacccgttatgccgacagcgttaagggccgtttcaccatttctgccgacacttccaagaacaccgcctacttgcagatgaactccttgagagccgaggatactgccgtctactactgcagccgttggggaggtgatgggttctacgccatggactactggggtcaaggcacccttgttaccgttagctccgccagcacaaagggtccctccgtcttccctttggctccctcctccaagtctacttccggtggtaccgctgcactgggttgcttggtcaaggactacttccctgagcccgtcactgtcagctggaattctggcgcattgacttctggtgtccacacttttcccgctgttctccaatcttccggcttgtacagcctaagcagcgttgtcactgtgccctcttcctccttgggcactcagacctacatctgcaacgtcaaccacaagccctccaacacgaaggttgacaagaaggtggaacctcccaagtcctgcgataagacccacacctgtcctccctgtcctgctcctgaactgttgggtggaccctcagtgttcttgttccctcccaagcccaaggacactctcatgatcagccgtactcctgaggttacatgcgtcgtcgtcgatgtctcccatgaggatcctgaggtcaagttcaactggtacgtcgacggtgtcgaggtccacaatgccaagaccaagcctcgtgaagaacagtacaactccacctaccgcgttgtttcagtcttgaccgtgttgcaccaggattggctgaacggcaaggagtacaagtgcaaggtctccaacaaggccctgcctgctcccatcgagaaaaccatcagtaaggccaaaggtcaacctcgcgaaccccaggtttacaccctccctccttctcgggacgaactcaccaagaaccaggtctcgttgacttgccttgttaagggattctaccctagcgatattgccgttgagtgggagtccaatggtcagcccgagaacaactacaagactacccctcctgttctcgactctgacggatctttcttcctctacagcaagttgaccgtcgacaaaagccgttggcagcaaggcaacgttttctcctgctctgtcatgcacgaggctctccacaaccactacacacagaagtctctgtccttgtctcctggtaaataa

SEQ ID NO: 66 - DNA, 1680 bp, Talaromyces cellulolyticus
attttcacttctttcttcgcctattgattgggctatgacaaaattaggagagataggttggacgttgtcaagtcaaaatgtaccgaacacgatgcgttgatatgctgcacatgtgcctagtatccattcgttcctatttatattaaattgaaattttcttatccaattactgagctaaaacatacttcagcactgtaagcgccagcctaagttatgctatgttagactgtccggattcggctggcactggcttttgtgatccccagtatcatgtaaaggtatccgcctgtttgttagggggtcttaaatgttgtataaagtttcttgctaggctgtttatgcttgatagagaatatatatatatatctagctgctattaatatccttgtttcaatgtcttagacttccaaggttacctacccgcgtgcgtggactaatacaaacaatctcactcaagacaatcttatacaaactcggattctggtcaatccgttccttggttatattgctaaaaaaactaggtagcccaaaattccatctcaagccgtataagaactttcaaattcaccatggtactctcacgggcgaagcatctccgtcttccatctgccaaaatccattaccaaaatcggaagtacccgaatgtagcaaatgaacaataactttcgcaccatctagcggatcctttgtgccacgatagttgttgaacgcagttttgcaatacccaggactaactgcttggatgataacactctcattcgccgggtctttcccatattcgaccgtgagcatgttaagggccgtctttgaggcgcagtacgcgatagtaacagttggaggcagcttgccagatgatgataggcccaaagaaccccgtgtggatgatacgtttattatgtggcctcgaggcgactgacgcaaaagtggtaggaatagatctatggtcattgcgaccgatgtgacattcacatcaaaagttcggttgtaagtagaccgcatttcggaaaatgaagtctgggtgaaggcaacggcagcattgtttatcagaactagacatctgttagagaatttctaaagcccgctcactcgagaatgaaataggcttaccatccagtctaccatatgttgtctcgaccgccttagcaaaagcaatgaggctatcgtcgcgagtcacatcaacctccataacgtcgatcttggattgaacagcgagctctctcaaccgcttaagtgcctgatttccgtcttccttattccggcatcctaagatgaagtgatcggatggactatgcagacttaaagcctggagggtaccaaacccgatgcctgacaattattagtgatcatatagaatgagtatcatggccatcgcaaatctacctctgtttgctccagttataagaattagccttgatgacatcttgtgagagaagtaaaagataatagcagatgaatttcgatcgtatactggttgtattggcaatcttgacgagaatggtttcattgtcagaccatcagttccctttatatacctgccattctctcctttataaataattattcggttttaacacggagatactcggatttcatcacacaaattgcatttcttccgatagttgttgaagatcggaagtccttcgaatgatcatttctataactacgccttaccgttttcgg

SEQ ID NO: 67 - DNA, 645 bp, Homo sapiens
gacatccagatgacacagtccccttctagcctttctgcctctgttggagatcgtgtcaccatcacttgtcgtgcttctcaagacgtcaacacagccgttgcctggtatcagcagaaacccggcaaagctcccaagttgctgatctacagcgctagcttcctgtacagcggtgtcccttctcgcttctcaggttcccgttctggtaccgacttcaccttgaccatttccagcttgcaacccgaggatttcgccacgtactactgccagcaacactacaccactcctcccacctttggccaaggtaccaaggtcgagatcaagcggactgttgccgcaccttccgtcttcatcttccctccctcggatgagcagctcaagtctggaactgcgtctgtcgtttgcttgctcaacaacttctaccctcgtgaagccaaggtccagtggaaggtcgacaacgctttgcagtccggcaatagccaagagtccgttaccgaacaggacagcaaggactccacttactccttgagttccactctcaccttgtccaaggccgattacgagaagcacaaggtctacgcttgcgaagtgacccatcaaggtctctctagccctgttactaagtccttcaaccgtggtgagtgttag

SEQ ID NO: 68 - DNA, 497 bp, Talaromyces cellulolyticus
atcagctttgagtgcagcaaaaatgcttccgactgtcttcttatattgatatcatatttttcaattcactttgtctcaagtttcaatatatcgagaaaatagtatcaaagatgaactgtaataattccgatatacctatacaggtttatagtaaattactctatttcataatgcgtccatccgagaagtctggcggccttatcagtagtccaaaacgcctggtttttagacatgtcacctctaatctccgcttgaggaaaatgcgtccgagcaagttctttcgacggggtgtcttgggtcgtagttggagatatgatatttattacttcgaatcctttgatattctcactcttttcaaccgccaaaaggcaagctcttgccactgcgcgaggattaacccatccccagagttgtcgaaccccagattcataccatttatcgtggtgtctttttctaacatctctcaatggggcaacctcatgtattctcaaacaagc

SEQ ID NO: 69 - DNA, 1812 bp, Talaromyces cellulolyticus
cactcaaccctatctcggtctattcttttgatttataagggattttgccgatttcggcctattggttaaaaaatgagctgatttaacaaaaatttaacgcgaattaattctgtggaatgtgtgtcagttagggtgtggaaagtccccaggctccccagcaggcagaagtatgcaaagcatgcatctcaattagtcagcaaccaggtgtggaaagtccccaggctccccagcaggcagaagtatgcaaagcatgcatctcaattagtcagcaaccatagtcccgcccctaactccgcccatcccgcccctaactccgcccagttccgcccattctccgccccatggctgactaattttttttatttatgcagaggccgaggccgcctctgcctctgagctattccagaagtagtgaggaggcttttttggaggcctaggcttttgcaaaaagctcccgggagcttgtatatccattttcggatctgatcagcacgtgatgaaaaagcctgaactcaccgcgacgtctgtcgagaagtttctgatcgaaaagttcgacagcgtctccgacctgatgcagctctcggagggcgaagaatctcgtgctttcagcttcgatgtaggagggcgtggatatgtcctgcgggtaaatagctgcgccgatggtttctacaaagatcgttatgtttatcggcactttgcatcggccgcgctcccgattccggaagtgcttgacattggggaattcagcgagagcctgacctattgcatctcccgccgtgcacagggtgtcacgttgcaagacctgcctgaaaccgaactgcccgctgttctgcagccggtcgcggaggccatggatgcgatcgctgcggccgatcttagccagacgagcgggttcggcccattcggaccgcaaggaatcggtcaatacactacatggcgtgatttcatatgcgcgattgctgatccccatgtgtatcactggcaaactgtgatggacgacaccgtcagtgcgtccgtcgcgcaggctctcgatgagctgatgctttgggccgaggactgccccgaagtccggcacctcgtgcacgcggatttcggctccaacaatgtcctgacggacaatggccgcataacagcggtcattgactggagcgaggcgatgttcggggattcccaatacgaggtcgccaacatcttcttctggaggccgtggttggcttgtatggagcagcagacgcgctacttcgagcggaggcatccggagcttgcaggatcgccgcggctccgggcgtatatgctccgcattggtcttgaccaactctatcagagcttggttgacggcaatttcgatgatgcagcttgggcgcagggtcgatgcgacgcaatcgtccgatccggagccgggactgtcgggcgtacacaaatcgcccgcagaagcgcggccgtctggaccgatggctgtgtagaagtactcgccgatagtggaaaccgacgccccagcactcgtccgagggcaaaggaatagcacgtgctacgagatttcgattccaccgccgccttctatgaaaggttgggcttcggaatcgttttccgggacgccggctggatgatcctccagcgcggggatctcatgctggagttcttcgcccaccccaacttgtttattgcagcttataatggttacaaataaagcaatagcatcacaaatttcacaaataaagcatttttttcactgcattctagttgtggtttgtccaaactcatcaatgtatcttatcatgtctgtataccgtcgacctctagctagagcttggc

SEQ ID NO: 70 - DNA, 1364 bp, Talaromyces cellulolyticus
atgaagactacctctgtgctcgcagccgccgcgctggccggcgctgctaccgccaaggtccacaagctcaagctggacaaggtgcctctctctgagcaatttgtatgacattctcaactcttcgctttaatttgtttctatggtcttgaactgatgatgatttgttaaaggataaacgcggcatgaacgaccacatgcggtctttgggtcagaagtacatgggcgttgtccccgagggaatgtaccaggacacctccatccgaccggagggcggccacgatgtgctggtcgataactttttgaacgctcagtgtatgtgaataccatcggatgatcttgatgatttgatgctaactattcgttctagacttctcagagatcaccatcggtacacccccacagaacttcaaggtcgtccttgataccgggagctcgaacttgtgggttccttcatcctcttgcaactcgattgcttgctacttgcacaacaagtatgactcgtcctcttcctctacctacaagaagaacggcagcgactttgccatccagtatggctcaggtagccttgagggcttcgtttcccgcgacactgtcacgattggcgacctttccattaaggaccaagacttcgccgaagccacaaacgagcctggcttggcttttgcctttggccgctttgacggtattttgggtcttggtttcgacaccatctcagtcaacaagattgtccctccgttctataacatgctaaaccagaagtctcttgatgagcctgtctttgccttctacctcggcgatagcaacaaggaaggtgatgattctgaggctacctttggtggtattgacgagagccactacactggaaagttggtcaagatccctctccgccgcaaggcctactgggaggtggactttgatgccattgcttttggcgacaacgttgctgagcttgagaacaccggagtcatccttgacactggtacttccctcattgctcttccttccactcttgccgagctcttgtaagtcatctattactcgctacacataaaaatatatgctaatatctttttaggaacaaggagattggtgcctccaagtcatggaacggtcaatacactgtcgactgtgccaagcgtgactctcttcccgacctcaccgtcaccctgagcggatacaacttctccatcagcgctttcgactacgttttggaagtccagggatcttgcatcagcgctttcatgggcatggacttccctgagcctgtcggccctcttgctatccttggtgatgctttcctccgcaagtggtacagcgtctacgacttgggcaacggtgccgtcggtctcgccaaggccaagtaa

SEQ ID NO: 71 - protein, 395 aa, Talaromyces cellulolyticus
MKTTSVLAAAALAGAATAKVHKLKLDKVPLSEQFDKRGMNDHMRSLGQKYMGVVPEGMYQDTSIRPEGGHDVLVDNFLNAQYFSEITIGTPPQNFKVVLDTGSSNLWVPSSSCNSIACYLHNKYDSSSSSTYKKNGSDFAIQYGSGSLEGFVSRDTVTIGDLSIKDQDFAEATNEPGLAFAFGRFDGILGLGFDTISVNKIVPPFYNMLNQKSLDEPVFAFYLGDSNKEGDDSEATFGGIDESHYTGKLVKIPLRRKAYWEVDFDAIAFGDNVAELENTGVILDTGTSLIALPSTLAELLNKEIGASKSWNGQYTVDCAKRDSLPDLTVTLSGYNFSISAFDYVLEVQGSCISAFMGMDFPEPVGPLAILGDAFLRKWYSVYDLGNGAVGLAKAK

SEQ ID NO: 72 - protein, 26 aa, Talaromyces cellulolyticus
MSALNSFNMYKSALILGSLLATAGAQ

SEQ ID NO: 73 - protein, 490 aa, Talaromyces cellulolyticus
MKGVLSLSLLPLLTVASPVMPRTIHNDAAPILSSSNAVEVPDSYIIVFKDHVDSASAAAHHNWVQDIHSQHTELRKRSQFPFADNAFAGLKHTFDIAGSFLGYSGHFEENVIEAIRRHPDVDYIEKDSLVHTMEDPALEKNAPWGLARISHRESLSFGSFNKYLYAADGGEGVDVYVIDTGTNIDHVDFEGRASWGKTIPTDDEDVDGNGHGTHCSGTIAGKKYGVAKKANVYAVKVLKSNGSGTMSDVVQGVEWAATQHIKKVKDAKAGKAKGFKGSAANMSLGGGKSVTLDKAVNAAVDAGIHFAVAAGNDNADSCNYSPAAAEKAVTVGASTLADERAYFSNYGKCNDIFAPGLNILSTWIGSKYAVNTISGTSMASPHIAGLLAYFLSLQPASDSAFAVAEITPKKLKENLIAIGTQGALTDVPSDTTNILAWNGGGSANYTDIIAQGGYKTKTLSNEVDELINKLEVVNEELGAIYSHIKDAIAA

SEQ ID NO: 74 - DNA, 4509 bp, Talaromyces cellulolyticus
atgtcgagaagaatacggaaccctgattccgcaggctcgagtcaaaccctaagtaattcaccggtaccaatagccgccgaatccggcacggaacctgtgtacctaggtccgtatcgaatagcgaagttttccgtctattcttcgaattttgtatacatgcttaccttggctcaaaggtactcacaaagtccgaagaataaattatagaaccgatgtgaaacggggacagtttggcaaccccttgtactatgtacattgtatggatctcgtctcgactctcgagacgagggtttcgtaccaaccaaagactcaaaacttggggtaactaagcgatcggctgcgtagtactccatactccataaataccccggtgaattcgcctcttgcccatggaatgagcgagaatttacccttggagtcatcgcggtaaatgactcacatatcatgtctgccttcactctcctcaacctttgaaattccggttaatgttaaggcgaggtgtcctctacggaatggctttgtagatttgagataagactacgccgtaacttaagggatccacatactccatattgatagtctcaggaccgagatagtctggagtaaccccgtacccaatcaacgtcctcagactcgccacctggttacaatatttcggtgcttgtgccgatatacctccgttgcgtgagccttgatagccaacaagaaatgattcaaaattaagatttgagaaaatccggagtacgcagtgcctgcagtgtaaaaaataatgtatttacctaatgccaatatgtcgatgccaaagtactactagcaaagacactagatatgcagcaaactcgatgtttaggtacatgtaaccatatcctggggtcaggtacgaacgccatcaattaatctcgtaaactagctgtcacacgacagtatcatttgatagttccaatgttccatgctccccctcaaatgtcactggatgatacgaatttggctgtgacttgaacagatagacggaaaacagtccgatcattatccggagtacgcatgtacgagatagtctggggatcctcggctgccccgattggggttagtgcgggtttccttatcttgatacgccgtctggaggcgcaggtgattgttacggtgtgttccgtgatagataagttagacatccgataataacctatcttctagatagacggcaggtacgtatgtagatagatagatgacacagtcataagacagttttatttaccatacatagtatagtcatttgacaaacacttgatgactatgagcagtaagtccagacaagagcatagactagaaatgatgtgatcatcaataggtacggagtcgtaccacccccggattatcttggctggcttagtcacgcccaaacagacggtgacggatgagacacaagcaaagagcgacattccgaagaattctcgtgacggaaacgagaatgccgccggcgctgatagggggaaattttatcttttccctttctgacattcagtgtttacaatacaatacggaattacggaaccccggttttcgcaaccggtggaattacctaatgggtgacctgaatttattagataacgatgaacaatttgttggatcttccgtagatcgatttggacttgataggtgcttccaaggttgttgctgctcacatggtcgcttgcgttatctgcctacagaatgaggaagatgtattccgcacgtactccggtcgcgacagatatgcgacgattgcaatatgtactacatagttagtacatacaactctagactagactctatattatgtagagtgtaagagaaaaagaaagaagataacggcagggtctatttgattgcgctataatatgcgccgctgtatggttccccagatctgcgtgagatatcacctcatcctatcatcattccaggtcaaagtctcgtcatcatgaattggtattattacccagtacgtaaaccacgtatcgaggcgtatcggtgtattaaagatagagctactgcattggctctagtcctatctttgccccggaatccggcccgtggatgacgatatgatgctgtttgtccttcagctaaacacggacgatctcttacagggtgcggttaattattaaggatataattctaatcaacgactctggctgtgctatattaacaatgtcttctaagtggtcatgatgtgtacgtacttcgtacacatgctacatgcaatcgagtacgtaactccagatctgcgccgtacccgcgatacccgggccatcatgcaaatgtaaccgcttggaacacgcactgcagtgcataaaagccacagcctcgcttcccaatccggtttagacgcgttttgtcttgctgttttgggagcagccagaccccacattccactaacccactctttttcagcgcttattctcgtaagattcgtacgaaaaatacatctgcccacactatccaccagctcggccactcttcggtgagaacgctgccatgagaaaaaaatctgcgactctgcaacagagtgaggcacggctgaaccgagctgattgtcaccctttgcccaatgcccagacagcccagacagcccagacagcccagacagcccagacagcccagacagcccagacagccagtgcttggttaatttttactaagggtaaaaacctaaaaaaaagaaacgaaaaaaaaaaaaaaaaacttttcttttttgccccccaatcacttggccgacagtcaaagggttcccccacacggtactccgtacttgctacgtacactaactaaagaaaaaatctcctgattgagtctgtgtctgtctgtcgctgctaaactcggataaccccccgttcccgatcacccgtcgaaaagagcagcagccatttaacatttttcccctccattcctccttcttggaactttccctccctccctcatccttacatctccctgcgtgcgcgcctgcctgcctacttacactgccactccccagattttctttctcttgtttcttctccagactttctttcctcctccacctcgcctcaccacaccaccaccaccactcaccacgccaacaacaccgcactaccactactgcttcaaagatcgatcaggccattatcaaggaggatcgacgtcttattccatcgaccaccctgttgatcacctcggctggagcgctcgactccctggcttccttccccagcttatttaaacccgtcacccgccaggtctcttcacatgtcaccgtcatcttcgtcagtgggtttttccaatctgctgaacccacagtcagactctgtcgagcctacggataacacatcttcacctgctaccaccactaccaccggcacagactccaactcagacaaggaaatggcgtcctctgtcagtctgctcccaccactcatgaagggtgcccgccccgccgcggaggaagtgcgacaggacctccctcgtccatacaagtgtcctctttgcgatcgtgctttccatcgtctagagcaccaaactcgtcacattcgtactcacaccggcgagaaaccccatgcctgccagtttccaggctgcacgaaacggttcagtcgttcagatgaattgactcgtcactcgcgcattcacaacaaccccaactcgagaagaagtaacaaagctcagcatattgctgcggctgcggcggccggtcaggattcgggtatgcttaacgctgctgcctcgatgatgcctcctccaagcaaacccattactcgctcggctccagtgtctcaggtcggatctccggatgtgtctcctccgcactcttacaccaactacacctcgcatttgcgggcgggtctgggtccttattcacgcaacagcgaccgtgcttcatctggtatggatattaatttgctcgcgactgctgcttcacaagtcgagcgcgatcactacggaggctcgtctcgtcattaccctttcagctctcgatactcgggtactcctggacgtctaccgtcgctttccgcctatgccatttctcagagcatgagccggtcgcattctcacgaggatgaggacaactacggacatcaccgggttaagcgctctcgtcctaactcaccaaactcgactgcgccatcctcgcctacattctctcacgattcattgtcgcctacccccgatcacactcctcttgcaaccccagcacactcgcctcgtttgcgtccttatggagccgcagatttgcaattaccttccatccgtcatttgtcgttacaccacactcccgcactcgcaccaatggagcctcaagccgagggacctaatgtttacaaccccggtcagcaccacggtggacccagcatcacggacatcatgagcaggcccgacggcacccagcgtaagcttcctgttccgcaagtacccaaaatcccggtgcaggacatgttggcaccgaacggatattcctccaacactccgtccgtcaacggttccgtgatggagttataa